European Patent Specification EP 4 022 052 B1, published July 1, 2026. Title: METHODS FOR PRODUCTION OF HUMAN RECOMBINANT ARGINASE 1 AND USES THEREOF. Applicant: Aeglea BioTherapeutics, Inc. The sequence listing filed with the application follows.

SEQUENCE LISTING (3 sequences)

SEQ ID NO: 1 - protein, 321 aa, Homo sapiens
SAKSRTIGIIGAPFSKGQPRGGVEEGPTVLRKAGLLEKLKEQECDVKDYGDLPFADIPNDSPFQIVKNPRSVGKASEQLAGKVAEVKKNGRISLVLGGDHSLAIGSISGHARVHPDLGVIWVDAHTDINTPLTTTSGNLHGQPVSFLLKELKGKIPDVPGFSWVTPCISAKDIVYIGLRDVDPGEHYILKTLGIKYFSMTEVDRLGIGKVMEETLSYLLGRKKRPIHLSFDVDGLDPSFTPATGTPVVGGLTYREGLYITEEIYKTGLLSGLDIMEVNPSLGKTPEEVTRTVNTAVAITLACFGLAREGNHKPIDYLNPPK

SEQ ID NO: 2 - DNA, 969 bp, Artificial Sequence
  Codon Optimized DNA Sequence
atgtctgcgaagagccgtacgatcggcattattggtgcgccgttctctaaaggtcagccacgcggtggtgtggaagagggtccgacggttctgcgtaaggccggtttattagaaaagctgaaagagcaggagtgcgacgttaaggactacggtgacttaccattcgcggacatcccgaatgatagcccgttccaaatcgttaagaatccgcgctctgtgggtaaagcaagcgagcagttagcaggtaaggtggccgaggtcaagaaaaacggtcgtattagcctggttttaggcggtgatcatagcttagcaattggctctatctctggtcatgcccgtgtgcacccagatttaggtgtcatttgggttgacgcccatacggatatcaatacgccattaacgaccaccagcggcaatctgcatggccagccggttagcttcttactgaaggagctgaagggtaaaattccagatgttccgggctttagctgggtcacgccatgtatttctgccaaggatatcgtgtacattggcttacgtgacgtcgacccaggtgagcactacatcttaaagaccctgggtatcaagtatttcagcatgacggaagtggaccgcttaggcatcggcaaggtgatggaggagacgctgagctatctgctgggccgtaagaaacgtccaatccatctgagcttcgatgttgacggcttagacccgagctttacgccagccaccggcacgccggtcgttggtggtttaacgtatcgcgaaggcctgtatatcacggaggaaatctataagacgggtttactgagcggtctggacattatggaggttaatccaagcttaggtaagacgccggaagaagttacccgtaccgttaacacggcggtcgcgatcacgttagcatgtttcggtttagcccgcgagggcaaccataaaccaattgattatctgaatccaccgaagtga

SEQ ID NO: 3 - protein, 353 aa, Homo sapiens
SLRGSLSRLLQTRVHSILKKSVHSVAVIGAPFSQGQKRKGVEHGPAAIREAGLMKRLSSLGCHLKDFGDLSFTPVPKDDLYNNLIVNPRSVGLANQELAEVVSRAVSDGYSCVTLGGDHSLAIGTISGHARHCPDLCVVWVDAHADINTPLTTSSGNLHGQPVSFLLRELQDKVPQLPGFSWIKPCISSASIVYIGLRDVDPPEHFILKNYDIQYFSMRDIDRLGIQKVMERTFDLLIGKRQRPIHLSFDIDAFDPTLAPATGTPVVGGLTYREGMYIAEEIHNTGLLSALDLVEVNPQLATSEEEAKTTANLAVDVIASSFGQTREGGHIVYDQLPTPSSPDESENQARVRI